European Patent Specification EP 4 034 661 B1, published September 6, 2023. Title: All-in-one AAV vectors for treating coronavirus induced diseases. Applicant: Georg-August-Universität Göttingen Stiftung Öffentlichen Rechts, Universitätsmedizin. The sequence listing filed with the application follows.

SEQUENCE LISTING (47 sequences)

SEQ ID NO: 1 - DNA, 27 bp, Artificial Sequence
  gRNA_XX-O-1
aacaattgtatgtgacaagtatttctt

SEQ ID NO: 2 - DNA, 27 bp, Artificial Sequence
  gRNA_XX-O-2
tacacgttcacctaagttggcgtatac

SEQ ID NO: 3 - DNA, 28 bp, Artificial Sequence
  gRNA_XX-O-3
agagaaagtgtgtctcttaactacaaag

SEQ ID NO: 4 - DNA, 28 bp, Artificial Sequence
  gRNA_XX-O-4
cgggtttgacagtttgaaaagcaacatt

SEQ ID NO: 5 - DNA, 27 bp, Artificial Sequence
  gRNA_XX-O-5
aatttgcttgttccaattactacagta

SEQ ID NO: 6 - DNA, 27 bp, Artificial Sequence
  gRNA_XX-O-6
ttaggataatcccaacccataaggtga

SEQ ID NO: 7 - DNA, 27 bp, Artificial Sequence
  gRNA_XX-O-7
tgcattaacattggccgtgacagcttg

SEQ ID NO: 8 - DNA, 27 bp, Artificial Sequence
  gRNA_XX-O-8
ctgtgtcaacatctctatttctataga

SEQ ID NO: 9 - DNA, 27 bp, Artificial Sequence
  gRNA_XX-O-9
acttaaagttctttatgctagccacta

SEQ ID NO: 10 - DNA, 27 bp, Artificial Sequence
  gRNA_XX-O-10
cattgagaaatgtttacgcaaatatgc

SEQ ID NO: 11 - DNA, 28 bp, Artificial Sequence
  gRNA_XX-O-11
agctctattctttgcactaatggcatac

SEQ ID NO: 12 - DNA, 28 bp, Artificial Sequence
  gRNA_XX-O-12
acaaatgttaaaaacactattagcataa

SEQ ID NO: 13 - DNA, 22 bp, Artificial Sequence
  gRNA_XX-O-13
gagctctattctttgcactaat

SEQ ID NO: 14 - DNA, 23 bp, Artificial Sequence
  gRNA_XX-O-14
gcatacttaagattcatttgagt

SEQ ID NO: 15 - DNA, 24 bp, Artificial Sequence
  gRNA_XX-O-15
actcttaccagtaccaggtggtcc

SEQ ID NO: 16 - DNA, 25 bp, Artificial Sequence
  gRNA_XX-O-16
cagcattaccatcctgagcaaagaa

SEQ ID NO: 17 - DNA, 22 bp, Artificial Sequence
  gRNA_XX-O-17
tgttgggtataagccagtaatt

SEQ ID NO: 18 - DNA, 23 bp, Artificial Sequence
  gRNA_XX-O-18
gagccctgtgatgaatcaacagt

SEQ ID NO: 19 - DNA, 27 bp, Artificial Sequence
  gRNA_XX-S-1
aaaacacttgaaattgcaccaaaattg

SEQ ID NO: 20 - DNA, 27 bp, Artificial Sequence
  gRNA_XX-S-2
agcctcaactttgtcaagacgtgaaag

SEQ ID NO: 21 - DNA, 27 bp, Artificial Sequence
  gRNA_XX-S-3
gcctgtgatcaacctatcaatttgcac

SEQ ID NO: 22 - DNA, 27 bp, Artificial Sequence
  gRNA_XX-S-4
tttgattgtccaagtacacactctgac

SEQ ID NO: 23 - DNA, 27 bp, Artificial Sequence
  gRNA_XX-E-1
tagtgtaactagcaagaataccacgaa

SEQ ID NO: 24 - DNA, 27 bp, Artificial Sequence
  gRNA_XX-E-2
acgcacacaatcgaagcgcagtaagga

SEQ ID NO: 25 - DNA, 27 bp, Artificial Sequence
  gRNA_XX-E-3
tttagaccagaagatcaggaactctag

SEQ ID NO: 26 - DNA, 27 bp, Artificial Sequence
  gRNA_XX-E-4
aataccacgaaagcaagaaaaagaagt

SEQ ID NO: 27 - DNA, 27 bp, Artificial Sequence
  gRNA_XX-M-1
gtaaacagcagcaagcacaaaacaagc

SEQ ID NO: 28 - DNA, 27 bp, Artificial Sequence
  gRNA_XX-M-2
gctgcgaagctcccaatttgtaataag

SEQ ID NO: 29 - DNA, 27 bp, Artificial Sequence
  gRNA_XX-N-1
tgggggcaaattgtgcaatttgcggcc

SEQ ID NO: 30 - DNA, 27 bp, Artificial Sequence
  gRNA_XX-N-2
tgaggaacgagaagaggcttgactgcc

SEQ ID NO: 31 - DNA, 22 bp, Artificial Sequence
  gRNA_XX-N-3
tcagcagcagatttcttagtga

SEQ ID NO: 32 - DNA, 22 bp, Artificial Sequence
  gRNA_Q-4-1
atatatgtggtaccatgtcacc

SEQ ID NO: 33 - DNA, 22 bp, Artificial Sequence
  gRNA_Q-4-2
attaccttcatcaaaatgcctt

SEQ ID NO: 34 - DNA, 22 bp, Artificial Sequence
  gRNA_Q-4-3
cttgattatctaatgtcagtac

SEQ ID NO: 35 - DNA, 22 bp, Artificial Sequence
  gRNA_Q-4-4
aagaatctacaacaggaactcc

SEQ ID NO: 36 - DNA, 22 bp, Artificial Sequence
  gRNA_Q-8-1
gaagaggcttgactgccgcctc

SEQ ID NO: 37 - DNA, 22 bp, Artificial Sequence
  gRNA_Q-8-2
gcctggagttgaatttcttgaa

SEQ ID NO: 38 - DNA, 22 bp, Artificial Sequence
  gRNA_Q-8-3
gttgttgttggcctttaccaga

SEQ ID NO: 39 - DNA, 22 bp, Artificial Sequence
  gRNA_Q-8-4
gcctcagcagcagatttcttag

SEQ ID NO: 40 - DNA, 7458 bp, Artificial Sequence
  pAAV-U6-gRNA-CMV-Cas13d
cctgcaggcagctgcgcgctcgctcgctcactgaggccgcccgggcgtcgggcgacctttggtcgcccggcctcagtgagcgagcgagcgcgcagagagggagtggccaactccatcactaggggttcctgcggccgcacgcgtaagcttgagggcctatttcccatgattccttcatatttgcatatacgatacaaggctgttagagagataattggaattaatttgactgtaaacacaaagatattagtacaaaatacgtgacgtagaaagtaataatttcttgggtagtttgcagttttaaaattatgttttaaaatggactatcatatgcttaccgtaacttgaaagtatttcgatttcttggctttatatatcttgtggaaaggacgaaacaccgaacccctaccaactggtcggggtttgaaactttttttgaattctgatgcggtattttctccttacgcatctgtgcggtatttcacaccgcatacgtcaaagcaaccatagtggtaccacgcgtggagctagttattaatagtaatcaattacggggtcattagttcatagcccatatatggagttccgcgttacataacttacggtaaatggcccgcctggctgaccgcccaacgacccccgcccattgacgtcaataatgacgtatgttcccatagtaacgtcaatagggactttccattgacgtcaatgggtggagtatttacggtaaactgcccacttggcagtacatcaagtgtatcatatgccaagtacgccccctattgacgtcaatgacggtaaatggcccgcctggcattatgcccagtacatgaccttatgggactttcctacttggcagtacatctacgtattagtcatcgctattaccatggtgatgcggttttggcagtacatcaatgggcgtggatagcggtttgactcacggggatttccaagtctccaccccattgacgtcaatgggagtttgttttgcaccaaaatcaacgggactttccaaaatgtcgtaacaactccgccccattgacgcaaatgggcggtaggcgtgtacggtgggaggtctatataagcagagctcgtttagtgaaccgtcagatcgcctggagacgccatccacgctgttttgacctccatagaagacaccgggaccgatccagcctccgcgggccaccatgagccccaagaagaagagaaaggtggaggccagcatcgaaaaaaaaaagtccttcgccaagggcatgggcgtgaagtccacactcgtgtccggctccaaagtgtacatgacaaccttcgccgaaggcagcgacgccaggctggaaaagatcgtggagggcgacagcatcaggagcgtgaatgagggcgaggccttcagcgctgaaatggccgataaaaacgccggctataagatcggcaacgccaaattcagccatcctaagggctacgccgtggtggctaacaaccctctgtatacaggacccgtccagcaggatatgctcggcctgaaggaaactctggaaaagaggtacttcggcgagagcgctgatggcaatgacaatatttgtatccaggtgatccataacatcctggacattgaaaaaatcctcgccgaatacattaccaacgccgcctacgccgtcaacaatatctccggcctggataaggacattattggattcggcaagttctccacagtgtatacctacgacgaattcaaagaccccgagcaccatagggccgctttcaacaataacgataagctcatcaacgccatcaaggcccagtatgacgagttcgacaacttcctcgataaccccagactcggctatttcggccaggcctttttcagcaaggagggcagaaattacatcatcaattacggcaacgaatgctatgacattctggccctcctgagcggactgaggcactgggtggtccataacaacgaagaagagtccaggatctccaggacctggctctacaacctcgataagaacctcgacaacgaatacatctccaccctcaactacctctacgacaggatcaccaatgagctgaccaactccttctccaagaactccgccgccaacgtgaactatattgccgaaactctgggaatcaaccctgccgaattcgccgaacaatatttcagattcagcattatgaaagagcagaaaaacctcggattcaatatcaccaagctcagggaagtgatgctggacaggaaggatatgtccgagatcaggaaaaatcataaggtgttcgactccatcaggaccaaggtctacaccatgatggactttgtgatttataggtattacatcgaagaggatgccaaggtggctgccgccaataagtccctccccgataatgagaagtccctgagcgagaaggatatctttgtgattaacctgaggggctccttcaacgacgaccagaaggatgccctctactacgatgaagctaatagaatttggagaaagctcgaaaatatcatgcacaacatcaaggaatttaggggaaacaagacaagagagtataagaagaaggacgcccctagactgcccagaatcctgcccgctggccgtgatgtttccgccttcagcaaactcatgtatgccctgaccatgttcctggatggcaaggagatcaacgacctcctgaccaccctgattaataaattcgataacatccagagcttcctgaaggtgatgcctctcatcggagtcaacgctaagttcgtggaggaatacgcctttttcaaagactccgccaagatcgccgatgagctgaggctgatcaagtccttcgctagaatgggagaacctattgccgatgccaggagggccatgtatatcgacgccatccgtattttaggaaccaacctgtcctatgatgagctcaaggccctcgccgacaccttttccctggacgagaacggaaacaagctcaagaaaggcaagcacggcatgagaaatttcattattaataacgtgatcagcaataaaaggttccactacctgatcagatacggtgatcctgcccacctccatgagatcgccaaaaacgaggccgtggtgaagttcgtgctcggcaggatcgctgacatccagaaaaaacagggccagaacggcaagaaccagatcgacaggtactacgaaacttgtatcggaaaggataagggcaagagcgtgagcgaaaaggtggacgctctcacaaagatcatcaccggaatgaactacgaccaattcgacaagaaaaggagcgtcattgaggacaccggcagggaaaacgccgagagggagaagtttaaaaagatcatcagcctgtacctcaccgtgatctaccacatcctcaagaatattgtcaatatcaacgccaggtacgtcatcggattccattgcgtcgagcgtgatgctcaactgtacaaggagaaaggctacgacatcaatctcaagaaactggaagagaagggattcagctccgtcaccaagctctgcgctggcattgatgaaactgcccccgataagagaaaggacgtggaaaaggagatggctgaaagagccaaggagagcattgacagcctcgagagcgccaaccccaagctgtatgccaattacatcaaatacagcgacgagaagaaagccgaggagttcaccaggcagattaacagggagaaggccaaaaccgccctgaacgcctacctgaggaacaccaagtggaatgtgatcatcagggaggacctcctgagaattgacaacaagacatgtaccctgttcagaaacaaggccgtccacctggaagtggccaggtatgtccacgcctatatcaacgacattgccgaggtcaattcctacttccaactgtaccattacatcatgcagagaattatcatgaatgagaggtacgagaaaagcagcggaaaggtgtccgagtacttcgacgctgtgaatgacgagaagaagtacaacgataggctcctgaaactgctgtgtgtgcctttcggctactgtatccccaggtttaagaacctgagcatcgaggccctgttcgataggaacgaggccgccaagttcgacaaggagaaaaagaaggtgtccggcaattccggatccggacctaagaaaaagaggaaggtggcggccgctgagcagaaactcatctcagaagaggatctgtaaagatctacgggtggcatccctgtgacccctccccagtgcctctcctggccctggaagttgccactccagtgcccaccagccttgtcctaataaaattaagttgcatcattttgtctgactaggtgtccttctataatattatggggtggaggggggtggtatggagcaaggggcaagttgggaagacaacctgtagggcctgcggggtctattgggaaccaagctggagtgcagtggcacaatcttggctcactgcaatctccgcctcctgggttcaagcgattctcctgcctcagcctcccgagttgttgggattccaggcatgcatgaccaggctcagctaatttttgtttttttggtagagacggggtttcaccatattggccaggctggtctccaactcctaatctcaggtgatctacccaccttggcctcccaaattgctgggattacaggcgtgaaccactgctcccttccctgtccttctgattttgtaggtaaccacgtgcggaccgagcggccgcaggaacccctagtgatggagttggccactccctctctgcgcgctcgctcgctcactgaggccgggcgaccaaaggtcgcccgacgcccgggctttgcccgggcggcctcagtgagcgagcgagcgcgcagctgcctgcaggggcgcctgatgcggtattttctccttacgcatctgtgcggtatttcacaccgcatacgtcaaagcaaccatagtacgcgccctgtagcggcgcattaagcgcggcgggtgtggtggttacgcgcagcgtgaccgctacacttgccagcgccctagcgcccgctcctttcgctttcttcccttcctttctcgccacgttcgccggctttccccgtcaagctctaaatcgggggctccctttagggttccgatttagtgctttacggcacctcgaccccaaaaaacttgatttgggtgatggttcacgtagtgggccatcgccctgatagacggtttttcgccctttgacgttggagtccacgttctttaatagtggactcttgttccaaactggaacaacactcaaccctatctcgggctattcttttgatttataagggattttgccgatttcggcctattggttaaaaaatgagctgatttaacaaaaatttaacgcgaattttaacaaaatattaacgtttacaattttatggtgcactctcagtacaatctgctctgatgccgcatagttaagccagccccgacacccgccaacacccgctgacgcgccctgacgggcttgtctgctcccggcatccgcttacagacaagctgtgaccgtctccgggagctgcatgtgtcagaggttttcaccgtcatcaccgaaacgcgcgagacgaaagggcctcgtgatacgcctatttttataggttaatgtcatgataataatggtttcttagacgtcaggtggcacttttcggggaaatgtgcgcggaacccctatttgtttatttttctaaatacattcaaatatgtatccgctcatgagacaataaccctgataaatgcttcaataatattgaaaaaggaagagtatgagtattcaacatttccgtgtcgcccttattcccttttttgcggcattttgccttcctgtttttgctcacccagaaacgctggtgaaagtaaaagatgctgaagatcagttgggtgcacgagtgggttacatcgaactggatctcaacagcggtaagatccttgagagttttcgccccgaagaacgttttccaatgatgagcacttttaaagttctgctatgtggcgcggtattatcccgtattgacgccgggcaagagcaactcggtcgccgcatacactattctcagaatgacttggttgagtactcaccagtcacagaaaagcatcttacggatggcatgacagtaagagaattatgcagtgctgccataaccatgagtgataacactgcggccaacttacttctgacaacgatcggaggaccgaaggagctaaccgcttttttgcacaacatgggggatcatgtaactcgccttgatcgttgggaaccggagctgaatgaagccataccaaacgacgagcgtgacaccacgatgcctgtagcaatggcaacaacgttgcgcaaactattaactggcgaactacttactctagcttcccggcaacaattaatagactggatggaggcggataaagttgcaggaccacttctgcgctcggcccttccggctggctggtttattgctgataaatctggagccggtgagcgtgggtctcgcggtatcattgcagcactggggccagatggtaagccctcccgtatcgtagttatctacacgacggggagtcaggcaactatggatgaacgaaatagacagatcgctgagataggtgcctcactgattaagcattggtaactgtcagaccaagtttactcatatatactttagattgatttaaaacttcatttttaatttaaaaggatctaggtgaagatcctttttgataatctcatgaccaaaatcccttaacgtgagttttcgttccactgagcgtcagaccccgtagaaaagatcaaaggatcttcttgagatcctttttttctgcgcgtaatctgctgcttgcaaacaaaaaaaccaccgctaccagcggtggtttgtttgccggatcaagagctaccaactctttttccgaaggtaactggcttcagcagagcgcagataccaaatactgtccttctagtgtagccgtagttaggccaccacttcaagaactctgtagcaccgcctacatacctcgctctgctaatcctgttaccagtggctgctgccagtggcgataagtcgtgtcttaccgggttggactcaagacgatagttaccggataaggcgcagcggtcgggctgaacggggggttcgtgcacacagcccagcttggagcgaacgacctacaccgaactgagatacctacagcgtgagctatgagaaagcgccacgcttcccgaagggagaaaggcggacaggtatccggtaagcggcagggtcggaacaggagagcgcacgagggagcttccagggggaaacgcctggtatctttatagtcctgtcgggtttcgccacctctgacttgagcgtcgatttttgtgatgctcgtcaggggggcggagcctatggaaaaacgccagcaacgcggcctttttacggttcctggccttttgctggccttttgctcacatgt

SEQ ID NO: 41 - DNA, 7669 bp, Artificial Sequence
  pAAV-U6-gRNA-CMV-Cas13d-array-triguide
cctgcaggcagctgcgcgctcgctcgctcactgaggccgcccgggcgtcgggcgacctttggtcgcccggcctcagtgagcgagcgagcgcgcagagagggagtggccaactccatcactaggggttcctgcggccgcacgcgtaagcttgagggcctatttcccatgattccttcatatttgcatatacgatacaaggctgttagagagataattggaattaatttgactgtaaacacaaagatattagtacaaaatacgtgacgtagaaagtaataatttcttgggtagtttgcagttttaaaattatgttttaaaatggactatcatatgcttaccgtaacttgaaagtatttcgatttcttggctttatatatcttgtggaaaggacgaaacaccgaacccctaccaactggtcggggtttgaaacgggaagagcgaactacacccgtgcaaaaatgcaggggtctaaaacgactgcaggtgggatcccacctgctcagatagcaatgaactacacccgtgcaaaaatgcaggggtctaaaacgggtcttcaagcttgaagacctatagcaatgaactacacccgtgcaaaaatgcaggggtctaaaaccgagacgtctagacgtctccgctcttcttttttttgaattctgatgcggtattttctccttacgcatctgtgcggtatttcacaccgcatacgtcaaagcaaccatagtggtaccacgcgtggagctagttattaatagtaatcaattacggggtcattagttcatagcccatatatggagttccgcgttacataacttacggtaaatggcccgcctggctgaccgcccaacgacccccgcccattgacgtcaataatgacgtatgttcccatagtaacgtcaatagggactttccattgacgtcaatgggtggagtatttacggtaaactgcccacttggcagtacatcaagtgtatcatatgccaagtacgccccctattgacgtcaatgacggtaaatggcccgcctggcattatgcccagtacatgaccttatgggactttcctacttggcagtacatctacgtattagtcatcgctattaccatggtgatgcggttttggcagtacatcaatgggcgtggatagcggtttgactcacggggatttccaagtctccaccccattgacgtcaatgggagtttgttttgcaccaaaatcaacgggactttccaaaatgtcgtaacaactccgccccattgacgcaaatgggcggtaggcgtgtacggtgggaggtctatataagcagagctcgtttagtgaaccgtcagatcgcctggagacgccatccacgctgttttgacctccatagaagacaccgggaccgatccagcctccgcgggccaccatgagccccaagaagaagagaaaggtggaggccagcatcgaaaaaaaaaagtccttcgccaagggcatgggcgtgaagtccacactcgtgtccggctccaaagtgtacatgacaaccttcgccgaaggcagcgacgccaggctggaaaagatcgtggagggcgacagcatcaggagcgtgaatgagggcgaggccttcagcgctgaaatggccgataaaaacgccggctataagatcggcaacgccaaattcagccatcctaagggctacgccgtggtggctaacaaccctctgtatacaggacccgtccagcaggatatgctcggcctgaaggaaactctggaaaagaggtacttcggcgagagcgctgatggcaatgacaatatttgtatccaggtgatccataacatcctggacattgaaaaaatcctcgccgaatacattaccaacgccgcctacgccgtcaacaatatctccggcctggataaggacattattggattcggcaagttctccacagtgtatacctacgacgaattcaaagaccccgagcaccatagggccgctttcaacaataacgataagctcatcaacgccatcaaggcccagtatgacgagttcgacaacttcctcgataaccccagactcggctatttcggccaggcctttttcagcaaggagggcagaaattacatcatcaattacggcaacgaatgctatgacattctggccctcctgagcggactgaggcactgggtggtccataacaacgaagaagagtccaggatctccaggacctggctctacaacctcgataagaacctcgacaacgaatacatctccaccctcaactacctctacgacaggatcaccaatgagctgaccaactccttctccaagaactccgccgccaacgtgaactatattgccgaaactctgggaatcaaccctgccgaattcgccgaacaatatttcagattcagcattatgaaagagcagaaaaacctcggattcaatatcaccaagctcagggaagtgatgctggacaggaaggatatgtccgagatcaggaaaaatcataaggtgttcgactccatcaggaccaaggtctacaccatgatggactttgtgatttataggtattacatcgaagaggatgccaaggtggctgccgccaataagtccctccccgataatgagaagtccctgagcgagaaggatatctttgtgattaacctgaggggctccttcaacgacgaccagaaggatgccctctactacgatgaagctaatagaatttggagaaagctcgaaaatatcatgcacaacatcaaggaatttaggggaaacaagacaagagagtataagaagaaggacgcccctagactgcccagaatcctgcccgctggccgtgatgtttccgccttcagcaaactcatgtatgccctgaccatgttcctggatggcaaggagatcaacgacctcctgaccaccctgattaataaattcgataacatccagagcttcctgaaggtgatgcctctcatcggagtcaacgctaagttcgtggaggaatacgcctttttcaaagactccgccaagatcgccgatgagctgaggctgatcaagtccttcgctagaatgggagaacctattgccgatgccaggagggccatgtatatcgacgccatccgtattttaggaaccaacctgtcctatgatgagctcaaggccctcgccgacaccttttccctggacgagaacggaaacaagctcaagaaaggcaagcacggcatgagaaatttcattattaataacgtgatcagcaataaaaggttccactacctgatcagatacggtgatcctgcccacctccatgagatcgccaaaaacgaggccgtggtgaagttcgtgctcggcaggatcgctgacatccagaaaaaacagggccagaacggcaagaaccagatcgacaggtactacgaaacttgtatcggaaaggataagggcaagagcgtgagcgaaaaggtggacgctctcacaaagatcatcaccggaatgaactacgaccaattcgacaagaaaaggagcgtcattgaggacaccggcagggaaaacgccgagagggagaagtttaaaaagatcatcagcctgtacctcaccgtgatctaccacatcctcaagaatattgtcaatatcaacgccaggtacgtcatcggattccattgcgtcgagcgtgatgctcaactgtacaaggagaaaggctacgacatcaatctcaagaaactggaagagaagggattcagctccgtcaccaagctctgcgctggcattgatgaaactgcccccgataagagaaaggacgtggaaaaggagatggctgaaagagccaaggagagcattgacagcctcgagagcgccaaccccaagctgtatgccaattacatcaaatacagcgacgagaagaaagccgaggagttcaccaggcagattaacagggagaaggccaaaaccgccctgaacgcctacctgaggaacaccaagtggaatgtgatcatcagggaggacctcctgagaattgacaacaagacatgtaccctgttcagaaacaaggccgtccacctggaagtggccaggtatgtccacgcctatatcaacgacattgccgaggtcaattcctacttccaactgtaccattacatcatgcagagaattatcatgaatgagaggtacgagaaaagcagcggaaaggtgtccgagtacttcgacgctgtgaatgacgagaagaagtacaacgataggctcctgaaactgctgtgtgtgcctttcggctactgtatccccaggtttaagaacctgagcatcgaggccctgttcgataggaacgaggccgccaagttcgacaaggagaaaaagaaggtgtccggcaattccggatccggacctaagaaaaagaggaaggtggcggccgctgagcagaaactcatctcagaagaggatctgtaaagatctacgggtggcatccctgtgacccctccccagtgcctctcctggccctggaagttgccactccagtgcccaccagccttgtcctaataaaattaagttgcatcattttgtctgactaggtgtccttctataatattatggggtggaggggggtggtatggagcaaggggcaagttgggaagacaacctgtagggcctgcggggtctattgggaaccaagctggagtgcagtggcacaatcttggctcactgcaatctccgcctcctgggttcaagcgattctcctgcctcagcctcccgagttgttgggattccaggcatgcatgaccaggctcagctaatttttgtttttttggtagagacggggtttcaccatattggccaggctggtctccaactcctaatctcaggtgatctacccaccttggcctcccaaattgctgggattacaggcgtgaaccactgctcccttccctgtccttctgattttgtaggtaaccacgtgcggaccgagcggccgcaggaacccctagtgatggagttggccactccctctctgcgcgctcgctcgctcactgaggccgggcgaccaaaggtcgcccgacgcccgggctttgcccgggcggcctcagtgagcgagcgagcgcgcagctgcctgcaggggcgcctgatgcggtattttctccttacgcatctgtgcggtatttcacaccgcatacgtcaaagcaaccatagtacgcgccctgtagcggcgcattaagcgcggcgggtgtggtggttacgcgcagcgtgaccgctacacttgccagcgccctagcgcccgctcctttcgctttcttcccttcctttctcgccacgttcgccggctttccccgtcaagctctaaatcgggggctccctttagggttccgatttagtgctttacggcacctcgaccccaaaaaacttgatttgggtgatggttcacgtagtgggccatcgccctgatagacggtttttcgccctttgacgttggagtccacgttctttaatagtggactcttgttccaaactggaacaacactcaaccctatctcgggctattcttttgatttataagggattttgccgatttcggcctattggttaaaaaatgagctgatttaacaaaaatttaacgcgaattttaacaaaatattaacgtttacaattttatggtgcactctcagtacaatctgctctgatgccgcatagttaagccagccccgacacccgccaacacccgctgacgcgccctgacgggcttgtctgctcccggcatccgcttacagacaagctgtgaccgtctccgggagctgcatgtgtcagaggttttcaccgtcatcaccgaaacgcgcgagacgaaagggcctcgtgatacgcctatttttataggttaatgtcatgataataatggtttcttagacgtcaggtggcacttttcggggaaatgtgcgcggaacccctatttgtttatttttctaaatacattcaaatatgtatccgctcatgagacaataaccctgataaatgcttcaataatattgaaaaaggaagagtatgagtattcaacatttccgtgtcgcccttattcccttttttgcggcattttgccttcctgtttttgctcacccagaaacgctggtgaaagtaaaagatgctgaagatcagttgggtgcacgagtgggttacatcgaactggatctcaacagcggtaagatccttgagagttttcgccccgaagaacgttttccaatgatgagcacttttaaagttctgctatgtggcgcggtattatcccgtattgacgccgggcaagagcaactcggtcgccgcatacactattctcagaatgacttggttgagtactcaccagtcacagaaaagcatcttacggatggcatgacagtaagagaattatgcagtgctgccataaccatgagtgataacactgcggccaacttacttctgacaacgatcggaggaccgaaggagctaaccgcttttttgcacaacatgggggatcatgtaactcgccttgatcgttgggaaccggagctgaatgaagccataccaaacgacgagcgtgacaccacgatgcctgtagcaatggcaacaacgttgcgcaaactattaactggcgaactacttactctagcttcccggcaacaattaatagactggatggaggcggataaagttgcaggaccacttctgcgctcggcccttccggctggctggtttattgctgataaatctggagccggtgagcgtgggtctcgcggtatcattgcagcactggggccagatggtaagccctcccgtatcgtagttatctacacgacggggagtcaggcaactatggatgaacgaaatagacagatcgctgagataggtgcctcactgattaagcattggtaactgtcagaccaagtttactcatatatactttagattgatttaaaacttcatttttaatttaaaaggatctaggtgaagatcctttttgataatctcatgaccaaaatcccttaacgtgagttttcgttccactgagcgtcagaccccgtagaaaagatcaaaggatcttcttgagatcctttttttctgcgcgtaatctgctgcttgcaaacaaaaaaaccaccgctaccagcggtggtttgtttgccggatcaagagctaccaactctttttccgaaggtaactggcttcagcagagcgcagataccaaatactgtccttctagtgtagccgtagttaggccaccacttcaagaactctgtagcaccgcctacatacctcgctctgctaatcctgttaccagtggctgctgccagtggcgataagtcgtgtcttaccgggttggactcaagacgatagttaccggataaggcgcagcggtcgggctgaacggggggttcgtgcacacagcccagcttggagcgaacgacctacaccgaactgagatacctacagcgtgagctatgagaaagcgccacgcttcccgaagggagaaaggcggacaggtatccggtaagcggcagggtcggaacaggagagcgcacgagggagcttccagggggaaacgcctggtatctttatagtcctgtcgggtttcgccacctctgacttgagcgtcgatttttgtgatgctcgtcaggggggcggagcctatggaaaaacgccagcaacgcggcctttttacggttcctggccttttgctggccttttgctcacatgt

SEQ ID NO: 42 - DNA, 7661 bp, Artificial Sequence
  pAAV-U6-quadguide-CMV-Cas13d-V3-basic
cctgcaggcagctgcgcgctcgctcgctcactgaggccgcccgggcgtcgggcgacctttggtcgcccggcctcagtgagcgagcgagcgcgcagagagggagtggccaactccatcactaggggttcctgcggccgcacgcgtaagcttgagggcctatttcccatgattccttcatatttgcatatacgatacaaggctgttagagagataattggaattaatttgactgtaaacacaaagatattagtacaaaatacgtgacgtagaaagtaataatttcttgggtagtttgcagttttaaaattatgttttaaaatggactatcatatgcttaccgtaacttgaaagtatttcgatttcttggctttatatatcttgtggaaaggacgaaacaccgaacccctaccaactggtcggggtttgaaacggaagagcgaaacaccgaacccctaccaactggtcggggtttgaaacgactgcaggtgggatcccacctgctcagagaaacaccgaacccctaccaactggtcggggtttgaaacgggtcttcaagcttgaagaccgaaacaccgaacccctaccaactggtcggggtttgaaaccgagacgtctagacgtctccgctcttcttttttttgaattctgatgcggtattttctccttacgcatctgtgcggtatttcacaccgcatacgtcaaagcaaccatagtggtaccacgcgtggagctagttattaatagtaatcaattacggggtcattagttcatagcccatatatggagttccgcgttacataacttacggtaaatggcccgcctggctgaccgcccaacgacccccgcccattgacgtcaataatgacgtatgttcccatagtaacgtcaatagggactttccattgacgtcaatgggtggagtatttacggtaaactgcccacttggcagtacatcaagtgtatcatatgccaagtacgccccctattgacgtcaatgacggtaaatggcccgcctggcattatgcccagtacatgaccttatgggactttcctacttggcagtacatctacgtattagtcatcgctattaccatggtgatgcggttttggcagtacatcaatgggcgtggatagcggtttgactcacggggatttccaagtctccaccccattgacgtcaatgggagtttgttttgcaccaaaatcaacgggactttccaaaatgtcgtaacaactccgccccattgacgcaaatgggcggtaggcgtgtacggtgggaggtctatataagcagagctcgtttagtgaaccgtcagatcgcctggagacgccatccacgctgttttgacctccatagaagacaccgggaccgatccagcctccgcgggccaccatgagccccaagaagaagagaaaggtggaggccagcatcgaaaaaaaaaagtccttcgccaagggcatgggcgtgaagtccacactcgtgtccggctccaaagtgtacatgacaaccttcgccgaaggcagcgacgccaggctggaaaagatcgtggagggcgacagcatcaggagcgtgaatgagggcgaggccttcagcgctgaaatggccgataaaaacgccggctataagatcggcaacgccaaattcagccatcctaagggctacgccgtggtggctaacaaccctctgtatacaggacccgtccagcaggatatgctcggcctgaaggaaactctggaaaagaggtacttcggcgagagcgctgatggcaatgacaatatttgtatccaggtgatccataacatcctggacattgaaaaaatcctcgccgaatacattaccaacgccgcctacgccgtcaacaatatctccggcctggataaggacattattggattcggcaagttctccacagtgtatacctacgacgaattcaaagaccccgagcaccatagggccgctttcaacaataacgataagctcatcaacgccatcaaggcccagtatgacgagttcgacaacttcctcgataaccccagactcggctatttcggccaggcctttttcagcaaggagggcagaaattacatcatcaattacggcaacgaatgctatgacattctggccctcctgagcggactgaggcactgggtggtccataacaacgaagaagagtccaggatctccaggacctggctctacaacctcgataagaacctcgacaacgaatacatctccaccctcaactacctctacgacaggatcaccaatgagctgaccaactccttctccaagaactccgccgccaacgtgaactatattgccgaaactctgggaatcaaccctgccgaattcgccgaacaatatttcagattcagcattatgaaagagcagaaaaacctcggattcaatatcaccaagctcagggaagtgatgctggacaggaaggatatgtccgagatcaggaaaaatcataaggtgttcgactccatcaggaccaaggtctacaccatgatggactttgtgatttataggtattacatcgaagaggatgccaaggtggctgccgccaataagtccctccccgataatgagaagtccctgagcgagaaggatatctttgtgattaacctgaggggctccttcaacgacgaccagaaggatgccctctactacgatgaagctaatagaatttggagaaagctcgaaaatatcatgcacaacatcaaggaatttaggggaaacaagacaagagagtataagaagaaggacgcccctagactgcccagaatcctgcccgctggccgtgatgtttccgccttcagcaaactcatgtatgccctgaccatgttcctggatggcaaggagatcaacgacctcctgaccaccctgattaataaattcgataacatccagagcttcctgaaggtgatgcctctcatcggagtcaacgctaagttcgtggaggaatacgcctttttcaaagactccgccaagatcgccgatgagctgaggctgatcaagtccttcgctagaatgggagaacctattgccgatgccaggagggccatgtatatcgacgccatccgtattttaggaaccaacctgtcctatgatgagctcaaggccctcgccgacaccttttccctggacgagaacggaaacaagctcaagaaaggcaagcacggcatgagaaatttcattattaataacgtgatcagcaataaaaggttccactacctgatcagatacggtgatcctgcccacctccatgagatcgccaaaaacgaggccgtggtgaagttcgtgctcggcaggatcgctgacatccagaaaaaacagggccagaacggcaagaaccagatcgacaggtactacgaaacttgtatcggaaaggataagggcaagagcgtgagcgaaaaggtggacgctctcacaaagatcatcaccggaatgaactacgaccaattcgacaagaaaaggagcgtcattgaggacaccggcagggaaaacgccgagagggagaagtttaaaaagatcatcagcctgtacctcaccgtgatctaccacatcctcaagaatattgtcaatatcaacgccaggtacgtcatcggattccattgcgtcgagcgtgatgctcaactgtacaaggagaaaggctacgacatcaatctcaagaaactggaagagaagggattcagctccgtcaccaagctctgcgctggcattgatgaaactgcccccgataagagaaaggacgtggaaaaggagatggctgaaagagccaaggagagcattgacagcctcgagagcgccaaccccaagctgtatgccaattacatcaaatacagcgacgagaagaaagccgaggagttcaccaggcagattaacagggagaaggccaaaaccgccctgaacgcctacctgaggaacaccaagtggaatgtgatcatcagggaggacctcctgagaattgacaacaagacatgtaccctgttcagaaacaaggccgtccacctggaagtggccaggtatgtccacgcctatatcaacgacattgccgaggtcaattcctacttccaactgtaccattacatcatgcagagaattatcatgaatgagaggtacgagaaaagcagcggaaaggtgtccgagtacttcgacgctgtgaatgacgagaagaagtacaacgataggctcctgaaactgctgtgtgtgcctttcggctactgtatccccaggtttaagaacctgagcatcgaggccctgttcgataggaacgaggccgccaagttcgacaaggagaaaaagaaggtgtccggcaattccggatccggacctaagaaaaagaggaaggtggcggccgctgagcagaaactcatctcagaagaggatctgtaaagatctacgggtggcatccctgtgacccctccccagtgcctctcctggccctggaagttgccactccagtgcccaccagccttgtcctaataaaattaagttgcatcattttgtctgactaggtgtccttctataatattatggggtggaggggggtggtatggagcaaggggcaagttgggaagacaacctgtagggcctgcggggtctattgggaaccaagctggagtgcagtggcacaatcttggctcactgcaatctccgcctcctgggttcaagcgattctcctgcctcagcctcccgagttgttgggattccaggcatgcatgaccaggctcagctaatttttgtttttttggtagagacggggtttcaccatattggccaggctggtctccaactcctaatctcaggtgatctacccaccttggcctcccaaattgctgggattacaggcgtgaaccactgctcccttccctgtccttctgattttgtaggtaaccacgtgcggaccgagcggccgcaggaacccctagtgatggagttggccactccctctctgcgcgctcgctcgctcactgaggccgggcgaccaaaggtcgcccgacgcccgggctttgcccgggcggcctcagtgagcgagcgagcgcgcagctgcctgcaggggcgcctgatgcggtattttctccttacgcatctgtgcggtatttcacaccgcatacgtcaaagcaaccatagtacgcgccctgtagcggcgcattaagcgcggcgggtgtggtggttacgcgcagcgtgaccgctacacttgccagcgccctagcgcccgctcctttcgctttcttcccttcctttctcgccacgttcgccggctttccccgtcaagctctaaatcgggggctccctttagggttccgatttagtgctttacggcacctcgaccccaaaaaacttgatttgggtgatggttcacgtagtgggccatcgccctgatagacggtttttcgccctttgacgttggagtccacgttctttaatagtggactcttgttccaaactggaacaacactcaaccctatctcgggctattcttttgatttataagggattttgccgatttcggcctattggttaaaaaatgagctgatttaacaaaaatttaacgcgaattttaacaaaatattaacgtttacaattttatggtgcactctcagtacaatctgctctgatgccgcatagttaagccagccccgacacccgccaacacccgctgacgcgccctgacgggcttgtctgctcccggcatccgcttacagacaagctgtgaccgtctccgggagctgcatgtgtcagaggttttcaccgtcatcaccgaaacgcgcgagacgaaagggcctcgtgatacgcctatttttataggttaatgtcatgataataatggtttcttagacgtcaggtggcacttttcggggaaatgtgcgcggaacccctatttgtttatttttctaaatacattcaaatatgtatccgctcatgagacaataaccctgataaatgcttcaataatattgaaaaaggaagagtatgagtattcaacatttccgtgtcgcccttattcccttttttgcggcattttgccttcctgtttttgctcacccagaaacgctggtgaaagtaaaagatgctgaagatcagttgggtgcacgagtgggttacatcgaactggatctcaacagcggtaagatccttgagagttttcgccccgaagaacgttttccaatgatgagcacttttaaagttctgctatgtggcgcggtattatcccgtattgacgccgggcaagagcaactcggtcgccgcatacactattctcagaatgacttggttgagtactcaccagtcacagaaaagcatcttacggatggcatgacagtaagagaattatgcagtgctgccataaccatgagtgataacactgcggccaacttacttctgacaacgatcggaggaccgaaggagctaaccgcttttttgcacaacatgggggatcatgtaactcgccttgatcgttgggaaccggagctgaatgaagccataccaaacgacgagcgtgacaccacgatgcctgtagcaatggcaacaacgttgcgcaaactattaactggcgaactacttactctagcttcccggcaacaattaatagactggatggaggcggataaagttgcaggaccacttctgcgctcggcccttccggctggctggtttattgctgataaatctggagccggtgagcgtgggtctcgcggtatcattgcagcactggggccagatggtaagccctcccgtatcgtagttatctacacgacggggagtcaggcaactatggatgaacgaaatagacagatcgctgagataggtgcctcactgattaagcattggtaactgtcagaccaagtttactcatatatactttagattgatttaaaacttcatttttaatttaaaaggatctaggtgaagatcctttttgataatctcatgaccaaaatcccttaacgtgagttttcgttccactgagcgtcagaccccgtagaaaagatcaaaggatcttcttgagatcctttttttctgcgcgtaatctgctgcttgcaaacaaaaaaaccaccgctaccagcggtggtttgtttgccggatcaagagctaccaactctttttccgaaggtaactggcttcagcagagcgcagataccaaatactgtccttctagtgtagccgtagttaggccaccacttcaagaactctgtagcaccgcctacatacctcgctctgctaatcctgttaccagtggctgctgccagtggcgataagtcgtgtcttaccgggttggactcaagacgatagttaccggataaggcgcagcggtcgggctgaacggggggttcgtgcacacagcccagcttggagcgaacgacctacaccgaactgagatacctacagcgtgagctatgagaaagcgccacgcttcccgaagggagaaaggcggacaggtatccggtaagcggcagggtcggaacaggagagcgcacgagggagcttccagggggaaacgcctggtatctttatagtcctgtcgggtttcgccacctctgacttgagcgtcgatttttgtgatgctcgtcaggggggcggagcctatggaaaaacgccagcaacgcggcctttttacggttcctggccttttgctggccttttgctcacatgt

SEQ ID NO: 43 - DNA, 7430 bp, Artificial Sequence
  pAAV-U6-gRNA-CMV-Cas13d-SapI
cctgcaggcagctgcgcgctcgctcgctcactgaggccgcccgggcgtcgggcgacctttggtcgcccggcctcagtgagcgagcgagcgcgcagagagggagtggccaactccatcactaggggttcctgcggccgcacgcgtaagcttgagggcctatttcccatgattccttcatatttgcatatacgatacaaggctgttagagagataattggaattaatttgactgtaaacacaaagatattagtacaaaatacgtgacgtagaaagtaataatttcttgggtagtttgcagttttaaaattatgttttaaaatggactatcatatgcttaccgtaacttgaaagtatttcgatttcttggctttatatatcttgtggaaaggacgaaacaccgaacccctaccaactggtcggggtttgaaacggaagagcgctagcagctcttcttttttttgaattctgatgcggtattttctccttacgcatctgtgcggtatttcacaccgcatacgtcaaagcaaccatagtggtaccacgcgtggagctagttattaatagtaatcaattacggggtcattagttcatagcccatatatggagttccgcgttacataacttacggtaaatggcccgcctggctgaccgcccaacgacccccgcccattgacgtcaataatgacgtatgttcccatagtaacgtcaatagggactttccattgacgtcaatgggtggagtatttacggtaaactgcccacttggcagtacatcaagtgtatcatatgccaagtacgccccctattgacgtcaatgacggtaaatggcccgcctggcattatgcccagtacatgaccttatgggactttcctacttggcagtacatctacgtattagtcatcgctattaccatggtgatgcggttttggcagtacatcaatgggcgtggatagcggtttgactcacggggatttccaagtctccaccccattgacgtcaatgggagtttgttttgcaccaaaatcaacgggactttccaaaatgtcgtaacaactccgccccattgacgcaaatgggcggtaggcgtgtacggtgggaggtctatataagcagagctcgtttagtgaaccgtcagatcgcctggagacgccatccacgctgttttgacctccatagaagacaccgggaccgatccagcctccgcgggccaccatgagcgaggccagcatcgaaaaaaaaaagtccttcgccaagggcatgggcgtgaagtccacactcgtgtccggctccaaagtgtacatgacaaccttcgccgaaggcagcgacgccaggctggaaaagatcgtggagggcgacagcatcaggagcgtgaatgagggcgaggccttcagcgctgaaatggccgataaaaacgccggctataagatcggcaacgccaaattcagccatcctaagggctacgccgtggtggctaacaaccctctgtatacaggacccgtccagcaggatatgctcggcctgaaggaaactctggaaaagaggtacttcggcgagagcgctgatggcaatgacaatatttgtatccaggtgatccataacatcctggacattgaaaaaatcctcgccgaatacattaccaacgccgcctacgccgtcaacaatatctccggcctggataaggacattattggattcggcaagttctccacagtgtatacctacgacgaattcaaagaccccgagcaccatagggccgctttcaacaataacgataagctcatcaacgccatcaaggcccagtatgacgagttcgacaacttcctcgataaccccagactcggctatttcggccaggcctttttcagcaaggagggcagaaattacatcatcaattacggcaacgaatgctatgacattctggccctcctgagcggactgaggcactgggtggtccataacaacgaagaagagtccaggatctccaggacctggctctacaacctcgataagaacctcgacaacgaatacatctccaccctcaactacctctacgacaggatcaccaatgagctgaccaactccttctccaagaactccgccgccaacgtgaactatattgccgaaactctgggaatcaaccctgccgaattcgccgaacaatatttcagattcagcattatgaaagagcagaaaaacctcggattcaatatcaccaagctcagggaagtgatgctggacaggaaggatatgtccgagatcaggaaaaatcataaggtgttcgactccatcaggaccaaggtctacaccatgatggactttgtgatttataggtattacatcgaagaggatgccaaggtggctgccgccaataagtccctccccgataatgagaagtccctgagcgagaaggatatctttgtgattaacctgaggggctccttcaacgacgaccagaaggatgccctctactacgatgaagctaatagaatttggagaaagctcgaaaatatcatgcacaacatcaaggaatttaggggaaacaagacaagagagtataagaagaaggacgcccctagactgcccagaatcctgcccgctggccgtgatgtttccgccttcagcaaactcatgtatgccctgaccatgttcctggatggcaaggagatcaacgacctcctgaccaccctgattaataaattcgataacatccagagcttcctgaaggtgatgcctctcatcggagtcaacgctaagttcgtggaggaatacgcctttttcaaagactccgccaagatcgccgatgagctgaggctgatcaagtccttcgctagaatgggagaacctattgccgatgccaggagggccatgtatatcgacgccatccgtattttaggaaccaacctgtcctatgatgagctcaaggccctcgccgacaccttttccctggacgagaacggaaacaagctcaagaaaggcaagcacggcatgagaaatttcattattaataacgtgatcagcaataaaaggttccactacctgatcagatacggtgatcctgcccacctccatgagatcgccaaaaacgaggccgtggtgaagttcgtgctcggcaggatcgctgacatccagaaaaaacagggccagaacggcaagaaccagatcgacaggtactacgaaacttgtatcggaaaggataagggcaagagcgtgagcgaaaaggtggacgctctcacaaagatcatcaccggaatgaactacgaccaattcgacaagaaaaggagcgtcattgaggacaccggcagggaaaacgccgagagggagaagtttaaaaagatcatcagcctgtacctcaccgtgatctaccacatcctcaagaatattgtcaatatcaacgccaggtacgtcatcggattccattgcgtcgagcgtgatgctcaactgtacaaggagaaaggctacgacatcaatctcaagaaactggaagagaagggattcagctccgtcaccaagctctgcgctggcattgatgaaactgcccccgataagagaaaggacgtggaaaaggagatggctgaaagagccaaggagagcattgacagcctcgagagcgccaaccccaagctgtatgccaattacatcaaatacagcgacgagaagaaagccgaggagttcaccaggcagattaacagggagaaggccaaaaccgccctgaacgcctacctgaggaacaccaagtggaatgtgatcatcagggaggacctcctgagaattgacaacaagacatgtaccctgttcagaaacaaggccgtccacctggaagtggccaggtatgtccacgcctatatcaacgacattgccgaggtcaattcctacttccaactgtaccattacatcatgcagagaattatcatgaatgagaggtacgagaaaagcagcggaaaggtgtccgagtacttcgacgctgtgaatgacgagaagaagtacaacgataggctcctgaaactgctgtgtgtgcctttcggctactgtatccccaggtttaagaacctgagcatcgaggccctgttcgataggaacgaggccgccaagttcgacaaggagaaaaagaaggtgtccggcaattccggatccggagagcagaaactcatctcagaagaggatctgtaaagatctacgggtggcatccctgtgacccctccccagtgcctctcctggccctggaagttgccactccagtgcccaccagccttgtcctaataaaattaagttgcatcattttgtctgactaggtgtccttctataatattatggggtggaggggggtggtatggagcaaggggcaagttgggaagacaacctgtagggcctgcggggtctattgggaaccaagctggagtgcagtggcacaatcttggctcactgcaatctccgcctcctgggttcaagcgattctcctgcctcagcctcccgagttgttgggattccaggcatgcatgaccaggctcagctaatttttgtttttttggtagagacggggtttcaccatattggccaggctggtctccaactcctaatctcaggtgatctacccaccttggcctcccaaattgctgggattacaggcgtgaaccactgctcccttccctgtccttctgattttgtaggtaaccacgtgcggaccgagcggccgcaggaacccctagtgatggagttggccactccctctctgcgcgctcgctcgctcactgaggccgggcgaccaaaggtcgcccgacgcccgggctttgcccgggcggcctcagtgagcgagcgagcgcgcagctgcctgcaggggcgcctgatgcggtattttctccttacgcatctgtgcggtatttcacaccgcatacgtcaaagcaaccatagtacgcgccctgtagcggcgcattaagcgcggcgggtgtggtggttacgcgcagcgtgaccgctacacttgccagcgccctagcgcccgctcctttcgctttcttcccttcctttctcgccacgttcgccggctttccccgtcaagctctaaatcgggggctccctttagggttccgatttagtgctttacggcacctcgaccccaaaaaacttgatttgggtgatggttcacgtagtgggccatcgccctgatagacggtttttcgccctttgacgttggagtccacgttctttaatagtggactcttgttccaaactggaacaacactcaaccctatctcgggctattcttttgatttataagggattttgccgatttcggcctattggttaaaaaatgagctgatttaacaaaaatttaacgcgaattttaacaaaatattaacgtttacaattttatggtgcactctcagtacaatctgctctgatgccgcatagttaagccagccccgacacccgccaacacccgctgacgcgccctgacgggcttgtctgctcccggcatccgcttacagacaagctgtgaccgtctccgggagctgcatgtgtcagaggttttcaccgtcatcaccgaaacgcgcgagacgaaagggcctcgtgatacgcctatttttataggttaatgtcatgataataatggtttcttagacgtcaggtggcacttttcggggaaatgtgcgcggaacccctatttgtttatttttctaaatacattcaaatatgtatccgctcatgagacaataaccctgataaatgcttcaataatattgaaaaaggaagagtatgagtattcaacatttccgtgtcgcccttattcccttttttgcggcattttgccttcctgtttttgctcacccagaaacgctggtgaaagtaaaagatgctgaagatcagttgggtgcacgagtgggttacatcgaactggatctcaacagcggtaagatccttgagagttttcgccccgaagaacgttttccaatgatgagcacttttaaagttctgctatgtggcgcggtattatcccgtattgacgccgggcaagagcaactcggtcgccgcatacactattctcagaatgacttggttgagtactcaccagtcacagaaaagcatcttacggatggcatgacagtaagagaattatgcagtgctgccataaccatgagtgataacactgcggccaacttacttctgacaacgatcggaggaccgaaggagctaaccgcttttttgcacaacatgggggatcatgtaactcgccttgatcgttgggaaccggagctgaatgaagccataccaaacgacgagcgtgacaccacgatgcctgtagcaatggcaacaacgttgcgcaaactattaactggcgaactacttactctagcttcccggcaacaattaatagactggatggaggcggataaagttgcaggaccacttctgcgctcggcccttccggctggctggtttattgctgataaatctggagccggtgagcgtgggtctcgcggtatcattgcagcactggggccagatggtaagccctcccgtatcgtagttatctacacgacggggagtcaggcaactatggatgaacgaaatagacagatcgctgagataggtgcctcactgattaagcattggtaactgtcagaccaagtttactcatatatactttagattgatttaaaacttcatttttaatttaaaaggatctaggtgaagatcctttttgataatctcatgaccaaaatcccttaacgtgagttttcgttccactgagcgtcagaccccgtagaaaagatcaaaggatcttcttgagatcctttttttctgcgcgtaatctgctgcttgcaaacaaaaaaaccaccgctaccagcggtggtttgtttgccggatcaagagctaccaactctttttccgaaggtaactggcttcagcagagcgcagataccaaatactgtccttctagtgtagccgtagttaggccaccacttcaagaactctgtagcaccgcctacatacctcgctctgctaatcctgttaccagtggctgctgccagtggcgataagtcgtgtcttaccgggttggactcaagacgatagttaccggataaggcgcagcggtcgggctgaacggggggttcgtgcacacagcccagcttggagcgaacgacctacaccgaactgagatacctacagcgtgagctatgagaaagcgccacgcttcccgaagggagaaaggcggacaggtatccggtaagcggcagggtcggaacaggagagcgcacgagggagcttccagggggaaacgcctggtatctttatagtcctgtcgggtttcgccacctctgacttgagcgtcgatttttgtgatgctcgtcaggggggcggagcctatggaaaaacgccagcaacgcggcctttttacggttcctggccttttgctggccttttgctcacatgt

SEQ ID NO: 44 - DNA, 7835 bp, Artificial Sequence
  pAAV-U6-gRNA-CMV-Cas13d-NTD-AarI
cctgcaggcagctgcgcgctcgctcgctcactgaggccgcccgggcgtcgggcgacctttggtcgcccggcctcagtgagcgagcgagcgcgcagagagggagtggccaactccatcactaggggttcctgcggccgcacgcgtaagcttgagggcctatttcccatgattccttcatatttgcatatacgatacaaggctgttagagagataattggaattaatttgactgtaaacacaaagatattagtacaaaatacgtgacgtagaaagtaataatttcttgggtagtttgcagttttaaaattatgttttaaaatggactatcatatgcttaccgtaacttgaaagtatttcgatttcttggctttatatatcttgtggaaaggacgaaacaccgaacccctaccaactggtcggggtttgaaacgactgcaggtggcgatcgccacctgctcagtttttttgaattctgatgcggtattttctccttacgcatctgtgcggtatttcacaccgcatacgtcaaagcaaccatagtggtaccacgcgtctagttattaatagtaatcaattacggggtcattagttcatagcccatatatggagttccgcgttacataacttacggtaaatggcccgcctggctgaccgcccaacgacccccgcccattgacgtcaataatgacgtatgttcccatagtaacgtcaatagggactttccattgacgtcaatgggtggagtatttacggtaaactgcccacttggcagtacatcaagtgtatcatatgccaagtacgccccctattgacgtcaatgacggtaaatggcccgcctggcattatgcccagtacatgaccttatgggactttcctacttggcagtacatctacgtattagtcatcgctattaccatggtgatgcggttttggcagtacatcaatgggcgtggatagcggtttgactcacggggatttccaagtctccaccccattgacgtcaatgggagtttgttttgcaccaaaatcaacgggactttccaaaatgtcgtaacaactccgccccattgacgcaaatgggcggtaggcgtgtacggtgggaggtctatataagcagagctcgtttagtgaaccgtcagatcgcctggagacgccatccacgctgttttgacctccatagaagacaccgggaccgatccagcctccgcgggccaccatgagcgaggccagcatcgaaaaaaaaaagtccttcgccaagggcatgggcgtgaagtccacactcgtgtccggctccaaagtgtacatgacaaccttcgccgaaggcagcgacgccaggctggaaaagatcgtggagggcgacagcatcaggagcgtgaatgagggcgaggccttcagcgctgaaatggccgataaaaacgccggctataagatcggcaacgccaaattcagccatcctaagggctacgccgtggtggctaacaaccctctgtatacaggacccgtccagcaggatatgctcggcctgaaggaaactctggaaaagaggtacttcggcgagagcgctgatggcaatgacaatatttgtatccaggtgatccataacatcctggacattgaaaaaatcctcgccgaatacattaccaacgccgcctacgccgtcaacaatatctccggcctggataaggacattattggattcggcaagttctccacagtgtatacctacgacgaattcaaagaccccgagcaccatagggccgctttcaacaataacgataagctcatcaacgccatcaaggcccagtatgacgagttcgacaacttcctcgataaccccagactcggctatttcggccaggcctttttcagcaaggagggcagaaattacatcatcaattacggcaacgaatgctatgacattctggccctcctgagcggactgaggcactgggtggtccataacaacgaagaagagtccaggatctccaggacctggctctacaacctcgataagaacctcgacaacgaatacatctccaccctcaactacctctacgacaggatcaccaatgagctgaccaactccttctccaagaactccgccgccaacgtgaactatattgccgaaactctgggaatcaaccctgccgaattcgccgaacaatatttcagattcagcattatgaaagagcagaaaaacctcggattcaatatcaccaagctcagggaagtgatgctggacaggaaggatatgtccgagatcaggaaaaatcataaggtgttcgactccatcaggaccaaggtctacaccatgatggactttgtgatttataggtattacatcgaagaggatgccaaggtggctgccgccaataagtccctccccgataatgagaagtccctgagcgagaaggatatctttgtgattaacctgaggggctccttcaacgacgaccagaaggatgccctctactacgatgaagctaatagaatttggagaaagctcgaaaatatcatgcacaacatcaaggaatttaggggaaacaagacaagagagtataagaagaaggacgcccctagactgcccagaatcctgcccgctggccgtgatgtttccgccttcagcaaactcatgtatgccctgaccatgttcctggatggcaaggagatcaacgacctcctgaccaccctgattaataaattcgataacatccagagcttcctgaaggtgatgcctctcatcggagtcaacgctaagttcgtggaggaatacgcctttttcaaagactccgccaagatcgccgatgagctgaggctgatcaagtccttcgctagaatgggagaacctattgccgatgccaggagggccatgtatatcgacgccatccgtattttaggaaccaacctgtcctatgatgagctcaaggccctcgccgacaccttttccctggacgagaacggaaacaagctcaagaaaggcaagcacggcatgagaaatttcattattaataacgtgatcagcaataaaaggttccactacctgatcagatacggtgatcctgcccacctccatgagatcgccaaaaacgaggccgtggtgaagttcgtgctcggcaggatcgctgacatccagaaaaaacagggccagaacggcaagaaccagatcgacaggtactacgaaacttgtatcggaaaggataagggcaagagcgtgagcgaaaaggtggacgctctcacaaagatcatcaccggaatgaactacgaccaattcgacaagaaaaggagcgtcattgaggacaccggcagggaaaacgccgagagggagaagtttaaaaagatcatcagcctgtacctcaccgtgatctaccacatcctcaagaatattgtcaatatcaacgccaggtacgtcatcggattccattgcgtcgagcgtgatgctcaactgtacaaggagaaaggctacgacatcaatctcaagaaactggaagagaagggattcagctccgtcaccaagctctgcgctggcattgatgaaactgcccccgataagagaaaggacgtggaaaaggagatggctgaaagagccaaggagagcattgacagcctcgagagcgccaaccccaagctgtatgccaattacatcaaatacagcgacgagaagaaagccgaggagttcaccaggcagattaacagggagaaggccaaaaccgccctgaacgcctacctgaggaacaccaagtggaatgtgatcatcagggaggacctcctgagaattgacaacaagacatgtaccctgttcagaaacaaggccgtccacctggaagtggccaggtatgtccacgcctatatcaacgacattgccgaggtcaattcctacttccaactgtaccattacatcatgcagagaattatcatgaatgagaggtacgagaaaagcagcggaaaggtgtccgagtacttcgacgctgtgaatgacgagaagaagtacaacgataggctcctgaaactgctgtgtgtgcctttcggctactgtatccccaggtttaagaacctgagcatcgaggccctgttcgataggaacgaggccgccaagttcgacaaggagaaaaagaaggtgtccggcaattcctctagaggcggaggcggatcgggccccaataatactgcgtcttggttcaccgctctcactcaacatggcaaggaagaccttaaattccctcgaggacaaggcgttccaattaacaccaatagcagtccagatgaccaaattggctactaccgaagagctaccagacgaattcgtggtggtgacggtaaaatgaaagatctcagtccaagatggtatttctactacctaggaactgggccagaagctggacttccctatggtgctaacaaagacggcatcatatgggttgcaactgagggagccttgaatacaccaaaagatcacattggcacccgcaatcctgctaacaatgctgcaatcgtgctacaacttcctcaaggaacaacattgccaaaaggcttctacgcagaagagcagaaactcatctcagaagaggatctgtaaagatctacgggtggcatccctgtgacccctccccagtgcctctcctggccctggaagttgccactccagtgcccaccagccttgtcctaataaaattaagttgcatcattttgtctgactaggtgtccttctataatattatggggtggaggggggtggtatggagcaaggggcaagttgggaagacaacctgtagggcctgcggggtctattgggaaccaagctggagtgcagtggcacaatcttggctcactgcaatctccgcctcctgggttcaagcgattctcctgcctcagcctcccgagttgttgggattccaggcatgcatgaccaggctcagctaatttttgtttttttggtagagacggggtttcaccatattggccaggctggtctccaactcctaatctcaggtgatctacccaccttggcctcccaaattgctgggattacaggcgtgaaccactgctcccttccctgtccttctgattttgtaggtaaccacgtgcggaccgagcggccgcaggaacccctagtgatggagttggccactccctctctgcgcgctcgctcgctcactgaggccgggcgaccaaaggtcgcccgacgcccgggctttgcccgggcggcctcagtgagcgagcgagcgcgcagctgcctgcaggggcgcctgatgcggtattttctccttacgcatctgtgcggtatttcacaccgcatacgtcaaagcaaccatagtacgcgccctgtagcggcgcattaagcgcggcgggtgtggtggttacgcgcagcgtgaccgctacacttgccagcgccctagcgcccgctcctttcgctttcttcccttcctttctcgccacgttcgccggctttccccgtcaagctctaaatcgggggctccctttagggttccgatttagtgctttacggcacctcgaccccaaaaaacttgatttgggtgatggttcacgtagtgggccatcgccctgatagacggtttttcgccctttgacgttggagtccacgttctttaatagtggactcttgttccaaactggaacaacactcaaccctatctcgggctattcttttgatttataagggattttgccgatttcggcctattggttaaaaaatgagctgatttaacaaaaatttaacgcgaattttaacaaaatattaacgtttacaattttatggtgcactctcagtacaatctgctctgatgccgcatagttaagccagccccgacacccgccaacacccgctgacgcgccctgacgggcttgtctgctcccggcatccgcttacagacaagctgtgaccgtctccgggagctgcatgtgtcagaggttttcaccgtcatcaccgaaacgcgcgagacgaaagggcctcgtgatacgcctatttttataggttaatgtcatgataataatggtttcttagacgtcaggtggcacttttcggggaaatgtgcgcggaacccctatttgtttatttttctaaatacattcaaatatgtatccgctcatgagacaataaccctgataaatgcttcaataatattgaaaaaggaagagtatgagtattcaacatttccgtgtcgcccttattcccttttttgcggcattttgccttcctgtttttgctcacccagaaacgctggtgaaagtaaaagatgctgaagatcagttgggtgcacgagtgggttacatcgaactggatctcaacagcggtaagatccttgagagttttcgccccgaagaacgttttccaatgatgagcacttttaaagttctgctatgtggcgcggtattatcccgtattgacgccgggcaagagcaactcggtcgccgcatacactattctcagaatgacttggttgagtactcaccagtcacagaaaagcatcttacggatggcatgacagtaagagaattatgcagtgctgccataaccatgagtgataacactgcggccaacttacttctgacaacgatcggaggaccgaaggagctaaccgcttttttgcacaacatgggggatcatgtaactcgccttgatcgttgggaaccggagctgaatgaagccataccaaacgacgagcgtgacaccacgatgcctgtagcaatggcaacaacgttgcgcaaactattaactggcgaactacttactctagcttcccggcaacaattaatagactggatggaggcggataaagttgcaggaccacttctgcgctcggcccttccggctggctggtttattgctgataaatctggagccggtgagcgtgggtctcgcggtatcattgcagcactggggccagatggtaagccctcccgtatcgtagttatctacacgacggggagtcaggcaactatggatgaacgaaatagacagatcgctgagataggtgcctcactgattaagcattggtaactgtcagaccaagtttactcatatatactttagattgatttaaaacttcatttttaatttaaaaggatctaggtgaagatcctttttgataatctcatgaccaaaatcccttaacgtgagttttcgttccactgagcgtcagaccccgtagaaaagatcaaaggatcttcttgagatcctttttttctgcgcgtaatctgctgcttgcaaacaaaaaaaccaccgctaccagcggtggtttgtttgccggatcaagagctaccaactctttttccgaaggtaactggcttcagcagagcgcagataccaaatactgtccttctagtgtagccgtagttaggccaccacttcaagaactctgtagcaccgcctacatacctcgctctgctaatcctgttaccagtggctgctgccagtggcgataagtcgtgtcttaccgggttggactcaagacgatagttaccggataaggcgcagcggtcgggctgaacggggggttcgtgcacacagcccagcttggagcgaacgacctacaccgaactgagatacctacagcgtgagctatgagaaagcgccacgcttcccgaagggagaaaggcggacaggtatccggtaagcggcagggtcggaacaggagagcgcacgagggagcttccagggggaaacgcctggtatctttatagtcctgtcgggtttcgccacctctgacttgagcgtcgatttttgtgatgctcgtcaggggggcggagcctatggaaaaacgccagcaacgcggcctttttacggttcctggccttttgctggccttttgctcacatgt

SEQ ID NO: 45 - DNA, 5064 bp, Artificial Sequence
  XX042f_pAAV-U6-quadguide-CMV-Cas13d-V3
cctgcaggcagctgcgcgctcgctcgctcactgaggccgcccgggcgtcgggcgacctttggtcgcccggcctcagtgagcgagcgagcgcgcagagagggagtggccaactccatcactaggggttcctgcggccgcacgcgtaagcttgagggcctatttcccatgattccttcatatttgcatatacgatacaaggctgttagagagataattggaattaatttgactgtaaacacaaagatattagtacaaaatacgtgacgtagaaagtaataatttcttgggtagtttgcagttttaaaattatgttttaaaatggactatcatatgcttaccgtaacttgaaagtatttcgatttcttggctttatatatcttgtggaaaggacgaaacaccgaacccctaccaactggtcggggtttgaaacggaagagcgaaacaccgaacccctaccaactggtcggggtttgaaacgactgcaggtgggatcccacctgctcagagaaacaccgaacccctaccaactggtcggggtttgaaacgggtcttcaagcttgaagaccgaaacaccgaacccctaccaactggtcggggtttgaaaccgagacgtctagacgtctccgctcttcttttttttgaattctgatgcggtattttctccttacgcatctgtgcggtatttcacaccgcatacgtcaaagcaaccatagtggtaccacgcgtggagctagttattaatagtaatcaattacggggtcattagttcatagcccatatatggagttccgcgttacataacttacggtaaatggcccgcctggctgaccgcccaacgacccccgcccattgacgtcaataatgacgtatgttcccatagtaacgtcaatagggactttccattgacgtcaatgggtggagtatttacggtaaactgcccacttggcagtacatcaagtgtatcatatgccaagtacgccccctattgacgtcaatgacggtaaatggcccgcctggcattatgcccagtacatgaccttatgggactttcctacttggcagtacatctacgtattagtcatcgctattaccatggtgatgcggttttggcagtacatcaatgggcgtggatagcggtttgactcacggggatttccaagtctccaccccattgacgtcaatgggagtttgttttgcaccaaaatcaacgggactttccaaaatgtcgtaacaactccgccccattgacgcaaatgggcggtaggcgtgtacggtgggaggtctatataagcagagctcgtttagtgaaccgtcagatcgcctggagacgccatccacgctgttttgacctccatagaagacaccgggaccgatccagcctccgcgggccaccatgagccccaagaagaagagaaaggtggaggccagcatcgaaaaaaaaaagtccttcgccaagggcatgggcgtgaagtccacactcgtgtccggctccaaagtgtacatgacaaccttcgccgaaggcagcgacgccaggctggaaaagatcgtggagggcgacagcatcaggagcgtgaatgagggcgaggccttcagcgctgaaatggccgataaaaacgccggctataagatcggcaacgccaaattcagccatcctaagggctacgccgtggtggctaacaaccctctgtatacaggacccgtccagcaggatatgctcggcctgaaggaaactctggaaaagaggtacttcggcgagagcgctgatggcaatgacaatatttgtatccaggtgatccataacatcctggacattgaaaaaatcctcgccgaatacattaccaacgccgcctacgccgtcaacaatatctccggcctggataaggacattattggattcggcaagttctccacagtgtatacctacgacgaattcaaagaccccgagcaccatagggccgctttcaacaataacgataagctcatcaacgccatcaaggcccagtatgacgagttcgacaacttcctcgataaccccagactcggctatttcggccaggcctttttcagcaaggagggcagaaattacatcatcaattacggcaacgaatgctatgacattctggccctcctgagcggactgaggcactgggtggtccataacaacgaagaagagtccaggatctccaggacctggctctacaacctcgataagaacctcgacaacgaatacatctccaccctcaactacctctacgacaggatcaccaatgagctgaccaactccttctccaagaactccgccgccaacgtgaactatattgccgaaactctgggaatcaaccctgccgaattcgccgaacaatatttcagattcagcattatgaaagagcagaaaaacctcggattcaatatcaccaagctcagggaagtgatgctggacaggaaggatatgtccgagatcaggaaaaatcataaggtgttcgactccatcaggaccaaggtctacaccatgatggactttgtgatttataggtattacatcgaagaggatgccaaggtggctgccgccaataagtccctccccgataatgagaagtccctgagcgagaaggatatctttgtgattaacctgaggggctccttcaacgacgaccagaaggatgccctctactacgatgaagctaatagaatttggagaaagctcgaaaatatcatgcacaacatcaaggaatttaggggaaacaagacaagagagtataagaagaaggacgcccctagactgcccagaatcctgcccgctggccgtgatgtttccgccttcagcaaactcatgtatgccctgaccatgttcctggatggcaaggagatcaacgacctcctgaccaccctgattaataaattcgataacatccagagcttcctgaaggtgatgcctctcatcggagtcaacgctaagttcgtggaggaatacgcctttttcaaagactccgccaagatcgccgatgagctgaggctgatcaagtccttcgctagaatgggagaacctattgccgatgccaggagggccatgtatatcgacgccatccgtattttaggaaccaacctgtcctatgatgagctcaaggccctcgccgacaccttttccctggacgagaacggaaacaagctcaagaaaggcaagcacggcatgagaaatttcattattaataacgtgatcagcaataaaaggttccactacctgatcagatacggtgatcctgcccacctccatgagatcgccaaaaacgaggccgtggtgaagttcgtgctcggcaggatcgctgacatccagaaaaaacagggccagaacggcaagaaccagatcgacaggtactacgaaacttgtatcggaaaggataagggcaagagcgtgagcgaaaaggtggacgctctcacaaagatcatcaccggaatgaactacgaccaattcgacaagaaaaggagcgtcattgaggacaccggcagggaaaacgccgagagggagaagtttaaaaagatcatcagcctgtacctcaccgtgatctaccacatcctcaagaatattgtcaatatcaacgccaggtacgtcatcggattccattgcgtcgagcgtgatgctcaactgtacaaggagaaaggctacgacatcaatctcaagaaactggaagagaagggattcagctccgtcaccaagctctgcgctggcattgatgaaactgcccccgataagagaaaggacgtggaaaaggagatggctgaaagagccaaggagagcattgacagcctcgagagcgccaaccccaagctgtatgccaattacatcaaatacagcgacgagaagaaagccgaggagttcaccaggcagattaacagggagaaggccaaaaccgccctgaacgcctacctgaggaacaccaagtggaatgtgatcatcagggaggacctcctgagaattgacaacaagacatgtaccctgttcagaaacaaggccgtccacctggaagtggccaggtatgtccacgcctatatcaacgacattgccgaggtcaattcctacttccaactgtaccattacatcatgcagagaattatcatgaatgagaggtacgagaaaagcagcggaaaggtgtccgagtacttcgacgctgtgaatgacgagaagaagtacaacgataggctcctgaaactgctgtgtgtgcctttcggctactgtatccccaggtttaagaacctgagcatcgaggccctgttcgataggaacgaggccgccaagttcgacaaggagaaaaagaaggtgtccggcaattccggatccggacctaagaaaaagaggaaggtggcggccgctgagcagaaactcatctcagaagaggatctgtaaagatctacgggtggcatccctgtgacccctccccagtgcctctcctggccctggaagttgccactccagtgcccaccagccttgtcctaataaaattaagttgcatcattttgtctgactaggtgtccttctataatattatggggtggaggggggtggtatggagcaaggggcaagttgggaagacaacctgtagggcctgcggggtctattgggaaccaagctggagtgcagtggcacaatcttggctcactgcaatctccgcctcctgggttcaagcgattctcctgcctcagcctcccgagttgttgggattccaggcatgcatgaccaggctcagctaatttttgtttttttggtagagacggggtttcaccatattggccaggctggtctccaactcctaatctcaggtgatctacccaccttggcctcccaaattgctgggattacaggcgtgaaccactgctcccttccctgtccttctgattttgtaggtaaccacgtgcggaccgagcggccgcaggaacccctagtgatggagttggccactccctctctgcgcgctcgctcgctcactgaggccgggcgaccaaaggtcgcccgacgcccgggctttgcccgggcggcctcagtgagcgagcgagcgcgcagctgcctgcagg

SEQ ID NO: 46 - DNA, 4833 bp, Artificial Sequence
  XX0042b_pAAV-U6-gRNA-CMV-Cas13d-SapI
cctgcaggcagctgcgcgctcgctcgctcactgaggccgcccgggcgtcgggcgacctttggtcgcccggcctcagtgagcgagcgagcgcgcagagagggagtggccaactccatcactaggggttcctgcggccgcacgcgtaagcttgagggcctatttcccatgattccttcatatttgcatatacgatacaaggctgttagagagataattggaattaatttgactgtaaacacaaagatattagtacaaaatacgtgacgtagaaagtaataatttcttgggtagtttgcagttttaaaattatgttttaaaatggactatcatatgcttaccgtaacttgaaagtatttcgatttcttggctttatatatcttgtggaaaggacgaaacaccgaacccctaccaactggtcggggtttgaaacggaagagcgctagcagctcttcttttttttgaattctgatgcggtattttctccttacgcatctgtgcggtatttcacaccgcatacgtcaaagcaaccatagtggtaccacgcgtggagctagttattaatagtaatcaattacggggtcattagttcatagcccatatatggagttccgcgttacataacttacggtaaatggcccgcctggctgaccgcccaacgacccccgcccattgacgtcaataatgacgtatgttcccatagtaacgtcaatagggactttccattgacgtcaatgggtggagtatttacggtaaactgcccacttggcagtacatcaagtgtatcatatgccaagtacgccccctattgacgtcaatgacggtaaatggcccgcctggcattatgcccagtacatgaccttatgggactttcctacttggcagtacatctacgtattagtcatcgctattaccatggtgatgcggttttggcagtacatcaatgggcgtggatagcggtttgactcacggggatttccaagtctccaccccattgacgtcaatgggagtttgttttgcaccaaaatcaacgggactttccaaaatgtcgtaacaactccgccccattgacgcaaatgggcggtaggcgtgtacggtgggaggtctatataagcagagctcgtttagtgaaccgtcagatcgcctggagacgccatccacgctgttttgacctccatagaagacaccgggaccgatccagcctccgcgggccaccatgagcgaggccagcatcgaaaaaaaaaagtccttcgccaagggcatgggcgtgaagtccacactcgtgtccggctccaaagtgtacatgacaaccttcgccgaaggcagcgacgccaggctggaaaagatcgtggagggcgacagcatcaggagcgtgaatgagggcgaggccttcagcgctgaaatggccgataaaaacgccggctataagatcggcaacgccaaattcagccatcctaagggctacgccgtggtggctaacaaccctctgtatacaggacccgtccagcaggatatgctcggcctgaaggaaactctggaaaagaggtacttcggcgagagcgctgatggcaatgacaatatttgtatccaggtgatccataacatcctggacattgaaaaaatcctcgccgaatacattaccaacgccgcctacgccgtcaacaatatctccggcctggataaggacattattggattcggcaagttctccacagtgtatacctacgacgaattcaaagaccccgagcaccatagggccgctttcaacaataacgataagctcatcaacgccatcaaggcccagtatgacgagttcgacaacttcctcgataaccccagactcggctatttcggccaggcctttttcagcaaggagggcagaaattacatcatcaattacggcaacgaatgctatgacattctggccctcctgagcggactgaggcactgggtggtccataacaacgaagaagagtccaggatctccaggacctggctctacaacctcgataagaacctcgacaacgaatacatctccaccctcaactacctctacgacaggatcaccaatgagctgaccaactccttctccaagaactccgccgccaacgtgaactatattgccgaaactctgggaatcaaccctgccgaattcgccgaacaatatttcagattcagcattatgaaagagcagaaaaacctcggattcaatatcaccaagctcagggaagtgatgctggacaggaaggatatgtccgagatcaggaaaaatcataaggtgttcgactccatcaggaccaaggtctacaccatgatggactttgtgatttataggtattacatcgaagaggatgccaaggtggctgccgccaataagtccctccccgataatgagaagtccctgagcgagaaggatatctttgtgattaacctgaggggctccttcaacgacgaccagaaggatgccctctactacgatgaagctaatagaatttggagaaagctcgaaaatatcatgcacaacatcaaggaatttaggggaaacaagacaagagagtataagaagaaggacgcccctagactgcccagaatcctgcccgctggccgtgatgtttccgccttcagcaaactcatgtatgccctgaccatgttcctggatggcaaggagatcaacgacctcctgaccaccctgattaataaattcgataacatccagagcttcctgaaggtgatgcctctcatcggagtcaacgctaagttcgtggaggaatacgcctttttcaaagactccgccaagatcgccgatgagctgaggctgatcaagtccttcgctagaatgggagaacctattgccgatgccaggagggccatgtatatcgacgccatccgtattttaggaaccaacctgtcctatgatgagctcaaggccctcgccgacaccttttccctggacgagaacggaaacaagctcaagaaaggcaagcacggcatgagaaatttcattattaataacgtgatcagcaataaaaggttccactacctgatcagatacggtgatcctgcccacctccatgagatcgccaaaaacgaggccgtggtgaagttcgtgctcggcaggatcgctgacatccagaaaaaacagggccagaacggcaagaaccagatcgacaggtactacgaaacttgtatcggaaaggataagggcaagagcgtgagcgaaaaggtggacgctctcacaaagatcatcaccggaatgaactacgaccaattcgacaagaaaaggagcgtcattgaggacaccggcagggaaaacgccgagagggagaagtttaaaaagatcatcagcctgtacctcaccgtgatctaccacatcctcaagaatattgtcaatatcaacgccaggtacgtcatcggattccattgcgtcgagcgtgatgctcaactgtacaaggagaaaggctacgacatcaatctcaagaaactggaagagaagggattcagctccgtcaccaagctctgcgctggcattgatgaaactgcccccgataagagaaaggacgtggaaaaggagatggctgaaagagccaaggagagcattgacagcctcgagagcgccaaccccaagctgtatgccaattacatcaaatacagcgacgagaagaaagccgaggagttcaccaggcagattaacagggagaaggccaaaaccgccctgaacgcctacctgaggaacaccaagtggaatgtgatcatcagggaggacctcctgagaattgacaacaagacatgtaccctgttcagaaacaaggccgtccacctggaagtggccaggtatgtccacgcctatatcaacgacattgccgaggtcaattcctacttccaactgtaccattacatcatgcagagaattatcatgaatgagaggtacgagaaaagcagcggaaaggtgtccgagtacttcgacgctgtgaatgacgagaagaagtacaacgataggctcctgaaactgctgtgtgtgcctttcggctactgtatccccaggtttaagaacctgagcatcgaggccctgttcgataggaacgaggccgccaagttcgacaaggagaaaaagaaggtgtccggcaattccggatccggagagcagaaactcatctcagaagaggatctgtaaagatctacgggtggcatccctgtgacccctccccagtgcctctcctggccctggaagttgccactccagtgcccaccagccttgtcctaataaaattaagttgcatcattttgtctgactaggtgtccttctataatattatggggtggaggggggtggtatggagcaaggggcaagttgggaagacaacctgtagggcctgcggggtctattgggaaccaagctggagtgcagtggcacaatcttggctcactgcaatctccgcctcctgggttcaagcgattctcctgcctcagcctcccgagttgttgggattccaggcatgcatgaccaggctcagctaatttttgtttttttggtagagacggggtttcaccatattggccaggctggtctccaactcctaatctcaggtgatctacccaccttggcctcccaaattgctgggattacaggcgtgaaccactgctcccttccctgtccttctgattttgtaggtaaccacgtgcggaccgagcggccgcaggaacccctagtgatggagttggccactccctctctgcgcgctcgctcgctcactgaggccgggcgaccaaaggtcgcccgacgcccgggctttgcccgggcggcctcagtgagcgagcgagcgcgcagctgcctgcagg

SEQ ID NO: 47 - DNA, 5238 bp, Artificial Sequence
  XX042d_pAAV-U6-gRNA-CMV-Cas13d-NTD-AarI
cctgcaggcagctgcgcgctcgctcgctcactgaggccgcccgggcgtcgggcgacctttggtcgcccggcctcagtgagcgagcgagcgcgcagagagggagtggccaactccatcactaggggttcctgcggccgcacgcgtaagcttgagggcctatttcccatgattccttcatatttgcatatacgatacaaggctgttagagagataattggaattaatttgactgtaaacacaaagatattagtacaaaatacgtgacgtagaaagtaataatttcttgggtagtttgcagttttaaaattatgttttaaaatggactatcatatgcttaccgtaacttgaaagtatttcgatttcttggctttatatatcttgtggaaaggacgaaacaccgaacccctaccaactggtcggggtttgaaacgactgcaggtggcgatcgccacctgctcagtttttttgaattctgatgcggtattttctccttacgcatctgtgcggtatttcacaccgcatacgtcaaagcaaccatagtggtaccacgcgtctagttattaatagtaatcaattacggggtcattagttcatagcccatatatggagttccgcgttacataacttacggtaaatggcccgcctggctgaccgcccaacgacccccgcccattgacgtcaataatgacgtatgttcccatagtaacgtcaatagggactttccattgacgtcaatgggtggagtatttacggtaaactgcccacttggcagtacatcaagtgtatcatatgccaagtacgccccctattgacgtcaatgacggtaaatggcccgcctggcattatgcccagtacatgaccttatgggactttcctacttggcagtacatctacgtattagtcatcgctattaccatggtgatgcggttttggcagtacatcaatgggcgtggatagcggtttgactcacggggatttccaagtctccaccccattgacgtcaatgggagtttgttttgcaccaaaatcaacgggactttccaaaatgtcgtaacaactccgccccattgacgcaaatgggcggtaggcgtgtacggtgggaggtctatataagcagagctcgtttagtgaaccgtcagatcgcctggagacgccatccacgctgttttgacctccatagaagacaccgggaccgatccagcctccgcgggccaccatgagcgaggccagcatcgaaaaaaaaaagtccttcgccaagggcatgggcgtgaagtccacactcgtgtccggctccaaagtgtacatgacaaccttcgccgaaggcagcgacgccaggctggaaaagatcgtggagggcgacagcatcaggagcgtgaatgagggcgaggccttcagcgctgaaatggccgataaaaacgccggctataagatcggcaacgccaaattcagccatcctaagggctacgccgtggtggctaacaaccctctgtatacaggacccgtccagcaggatatgctcggcctgaaggaaactctggaaaagaggtacttcggcgagagcgctgatggcaatgacaatatttgtatccaggtgatccataacatcctggacattgaaaaaatcctcgccgaatacattaccaacgccgcctacgccgtcaacaatatctccggcctggataaggacattattggattcggcaagttctccacagtgtatacctacgacgaattcaaagaccccgagcaccatagggccgctttcaacaataacgataagctcatcaacgccatcaaggcccagtatgacgagttcgacaacttcctcgataaccccagactcggctatttcggccaggcctttttcagcaaggagggcagaaattacatcatcaattacggcaacgaatgctatgacattctggccctcctgagcggactgaggcactgggtggtccataacaacgaagaagagtccaggatctccaggacctggctctacaacctcgataagaacctcgacaacgaatacatctccaccctcaactacctctacgacaggatcaccaatgagctgaccaactccttctccaagaactccgccgccaacgtgaactatattgccgaaactctgggaatcaaccctgccgaattcgccgaacaatatttcagattcagcattatgaaagagcagaaaaacctcggattcaatatcaccaagctcagggaagtgatgctggacaggaaggatatgtccgagatcaggaaaaatcataaggtgttcgactccatcaggaccaaggtctacaccatgatggactttgtgatttataggtattacatcgaagaggatgccaaggtggctgccgccaataagtccctccccgataatgagaagtccctgagcgagaaggatatctttgtgattaacctgaggggctccttcaacgacgaccagaaggatgccctctactacgatgaagctaatagaatttggagaaagctcgaaaatatcatgcacaacatcaaggaatttaggggaaacaagacaagagagtataagaagaaggacgcccctagactgcccagaatcctgcccgctggccgtgatgtttccgccttcagcaaactcatgtatgccctgaccatgttcctggatggcaaggagatcaacgacctcctgaccaccctgattaataaattcgataacatccagagcttcctgaaggtgatgcctctcatcggagtcaacgctaagttcgtggaggaatacgcctttttcaaagactccgccaagatcgccgatgagctgaggctgatcaagtccttcgctagaatgggagaacctattgccgatgccaggagggccatgtatatcgacgccatccgtattttaggaaccaacctgtcctatgatgagctcaaggccctcgccgacaccttttccctggacgagaacggaaacaagctcaagaaaggcaagcacggcatgagaaatttcattattaataacgtgatcagcaataaaaggttccactacctgatcagatacggtgatcctgcccacctccatgagatcgccaaaaacgaggccgtggtgaagttcgtgctcggcaggatcgctgacatccagaaaaaacagggccagaacggcaagaaccagatcgacaggtactacgaaacttgtatcggaaaggataagggcaagagcgtgagcgaaaaggtggacgctctcacaaagatcatcaccggaatgaactacgaccaattcgacaagaaaaggagcgtcattgaggacaccggcagggaaaacgccgagagggagaagtttaaaaagatcatcagcctgtacctcaccgtgatctaccacatcctcaagaatattgtcaatatcaacgccaggtacgtcatcggattccattgcgtcgagcgtgatgctcaactgtacaaggagaaaggctacgacatcaatctcaagaaactggaagagaagggattcagctccgtcaccaagctctgcgctggcattgatgaaactgcccccgataagagaaaggacgtggaaaaggagatggctgaaagagccaaggagagcattgacagcctcgagagcgccaaccccaagctgtatgccaattacatcaaatacagcgacgagaagaaagccgaggagttcaccaggcagattaacagggagaaggccaaaaccgccctgaacgcctacctgaggaacaccaagtggaatgtgatcatcagggaggacctcctgagaattgacaacaagacatgtaccctgttcagaaacaaggccgtccacctggaagtggccaggtatgtccacgcctatatcaacgacattgccgaggtcaattcctacttccaactgtaccattacatcatgcagagaattatcatgaatgagaggtacgagaaaagcagcggaaaggtgtccgagtacttcgacgctgtgaatgacgagaagaagtacaacgataggctcctgaaactgctgtgtgtgcctttcggctactgtatccccaggtttaagaacctgagcatcgaggccctgttcgataggaacgaggccgccaagttcgacaaggagaaaaagaaggtgtccggcaattcctctagaggcggaggcggatcgggccccaataatactgcgtcttggttcaccgctctcactcaacatggcaaggaagaccttaaattccctcgaggacaaggcgttccaattaacaccaatagcagtccagatgaccaaattggctactaccgaagagctaccagacgaattcgtggtggtgacggtaaaatgaaagatctcagtccaagatggtatttctactacctaggaactgggccagaagctggacttccctatggtgctaacaaagacggcatcatatgggttgcaactgagggagccttgaatacaccaaaagatcacattggcacccgcaatcctgctaacaatgctgcaatcgtgctacaacttcctcaaggaacaacattgccaaaaggcttctacgcagaagagcagaaactcatctcagaagaggatctgtaaagatctacgggtggcatccctgtgacccctccccagtgcctctcctggccctggaagttgccactccagtgcccaccagccttgtcctaataaaattaagttgcatcattttgtctgactaggtgtccttctataatattatggggtggaggggggtggtatggagcaaggggcaagttgggaagacaacctgtagggcctgcggggtctattgggaaccaagctggagtgcagtggcacaatcttggctcactgcaatctccgcctcctgggttcaagcgattctcctgcctcagcctcccgagttgttgggattccaggcatgcatgaccaggctcagctaatttttgtttttttggtagagacggggtttcaccatattggccaggctggtctccaactcctaatctcaggtgatctacccaccttggcctcccaaattgctgggattacaggcgtgaaccactgctcccttccctgtccttctgattttgtaggtaaccacgtgcggaccgagcggccgcaggaacccctagtgatggagttggccactccctctctgcgcgctcgctcgctcactgaggccgggcgaccaaaggtcgcccgacgcccgggctttgcccgggcggcctcagtgagcgagcgagcgcgcagctgcctgcagg